European Patent Specification EP 3 596 226 B1, published April 23, 2025. Title: Oligosaccharyltransferase Polypeptide. Applicant: London School of Hygiene & Tropical Medicine. The sequence listing filed with the application follows.

SEQUENCE LISTING (45 sequences)

SEQ ID NO: 1 - DNA, 2133 bp, Campylobacter sputorum
atgtcaaattttaatttcgctaaatttctaaataaattacctagactttctaaacatactatattaatgattgttttagctgtttgttttgggatattttgcagattttactgggtagtttgggctagtgcttatccccattttatatggaatgatgaacttatgataagtacaaatgatggatatgcatttgctgagggcacaagagatatgatagctggttttcatcaaccaaacgatctttcttactatggctcatctctttctacacttagcatgtggctatatagcattttgccattttcattagaaactatacttttgtatatgagtacatttttatctccactattagctgtgcctttgatacttataggtaaagaactaaacgcttcaaaagctggatttatagctgcacttctagctgttgttgcaaatagttattataatagaacaatgagtggatattatgatacagatatgctaaatattactcttcctatgatggttttttggagcataacaagacttgttcaaagaaaagagagagtaaatttaatatttattccagtttttatggcgatatatggatggtggtatccatcttcttactcactattactcgcaatgattgggatgtttgttttatataccattgtttttgaaagatatgaaaaactaaactatgaagctatggtttttatgattttggcaatcacaagctttcctatacaaatcaaatttattatagttattattttgtatgctttgatctatttttatcaaagattttttgataaaaaagtaatatttgcattaattatagcttcatcaatatgctttatatggcttggcggattaaatcctatactttttaacattaaattttatatatttagagacattgcagatagtggtgatactgtttttaaatttttcaatgtaaatcaaacaataagagaaagttccgcgatagattttaatacagttgcaactaggattagtgggcatttgatagtatttttggtatctattgtaggatatattttatttataaaaaacaataaaattttactactaactttaccgattctatttttaggtcttatgtcatttaaaagtggtttaagatttacaatatactcagttccagtaatggcccttggttttggttattttgttatgtattgttttacaaagatagatataaaagatcgttttttaggttatgcatttttatttgttgtaacatttagtgcattatatccatctttaaaacatatttatgattataaggtatttcctgtttttacacatagcgaagttgaaagtttggatgatttaaaaaatattgcaaaaagagaagattatgtgctttcttggtgggattatggttatccaataagatattattctgatgtaaaaactctcatagatggaggaaaacatctaggaagtgataacttcgcagttagctttgcacttggaagcgatcaaaacagctctgcaaatatggcaagattagaagttgagtatacagaaagaaattatgaggaaaaatttggattaaatttaaaacagattatgaaagattataatgctacaaatgttaatgagtttttattatcattaaaagatgcaaatttagctctgccaaagcaaacaagagatatttattactatttaccagatagaatgatatacatatatccaacagtgctagctttttctagacttgatttgacaacagggcaagaatttgctgagccgttttttatagttagtgagagattttcagctacaaatgataatcaaataatgttaaataataatgttatattaagtagtgatggcactaaattatcaataaatggaaactcttatagtgtaaatacatatgtagaaacaagttatgatcaaaatgaaaaattaaatgtaaattattttaacatagatccaaatagcaatttttatgtgatttttatgaaagattatttgagaattttggttttagataaaactttatatgatagtgcgtatattcaactttttgtattagaaaattatgataaaaatttatttgaaccagtgattttaaacggatcaactaaaatttataaactcaaaaaatga

SEQ ID NO: 2 - DNA, 2133 bp, Campylobacter sputorum
atgagtaattttaattttgccaaatttctgaacaagctgcctagactaagcaaacataccatcctgatgatcgtgctggcggtgtgctttggcatcttttgtcgcttttattgggttgtgtgggcgagtgcgtatccacattttatttggaatgatgaactgatgatctctacaaatgatggctatgcgtttgcggaaggtacacgcgatatgattgccggctttcatcagccgaatgatctgtcatattatggtagttcactgtccactttaagcatgtggctgtatagcatcctgccgttttcattagaaaccatcttactgtatatgtcaacgtttctgagtccactgctggcagttccgttaatcttaatcggtaaagaactgaatgcgtctaaagcaggctttattgcagccctgctggcagttgtggccaatagctattataatcgcaccatgtcaggctattatgatacggatatgctgaatatcaccttaccgatgatggtgttttggagcatcacccgcctggttcagcgcaaagaacgggttaatctcatctttattccagtgtttatggccatctatggttggtggtatccatcttcatattcactgctgctggccatgatcggcatgtttgtgctgtataccatcgtgtttgaacgctatgaaaaactgaattatgaagcaatggtgtttatgattctggcaatcactagctttccgattcagatcaagtttatcatcgtgatcattctgtatgcgttaatctatttttatcagcgctttttcgataaaaaagttatctttgccttaatcattgcaagtagcatttgctttatttggttaggcggcttaaatccaatcctgtttaatatcaaattttatatctttcgcgacatagcggattcaggcgatacggtgtttaaattcttcaatgtgaatcagaccattcgcgaaagtagcgccatcgattttaatacagttgcgacccgcatctcaggtcatctgattgtgtttctggtgagcatcgtgggctatatcctgtttatcaaaaacaacaagattttactgctgaccttaccgatcctgtttctgggtctgatgtcgtttaaaagcggcctgcgctttacaatctatagcgttcctgtaatggcgttaggctttggctattttgtgatgtattgctttacgaaaatcgacatcaaagatcgctttctgggctatgcctttctgtttgtggtgacctttagtgccctgtatccgtcactgaaacatatctatgattacaaggtgtttccagtgtttacacatagcgaagtggaaagcctggatgatctgaaaaatattgccaaacgcgaagattatgtgctgtcttggtgggattatggctatccgattcgctattatagcgatgttaaaacactgatcgatggcggtaaacatctaggttcagataattttgccgtgagctttgcactgggcagcgatcagaatagtagtgcaaatatggcccgcttagaagtggaatatacggaacgcaattatgaagaaaaatttggtctgaatctgaaacagatcatgaaagattataatgcaaccaatgtgaatgagtttctgctgtctctgaaagatgccaacctggccctgcctaaacagacacgcgatatatattattatctgccggatcgcatgatctatatctatcctacagtgttagcctttagtcgcctggatctgacgacgggccaggaatttgcagaaccgtttttcatcgtgagcgaacgctttagtgcaaccaatgataatcagatcatgttaaacaacaatgtgattctttcatcagatggaacaaaactgtcaatcaatggcaatagctattcagttaatacttatgtagaaaccagctacgatcagaacgaaaaactgaatgttaattattttaatatcgatccgaatagcaatttttatgtgatctttatgaaagattatctgcgcatcttagttctggataaaaccctgtatgatagcgcgtatatccagctgtttgtgctggaaaattatgataaaaatctgtttgaaccagtcatcctgaatggtagtacgaaaatctataagctgaaaaaataa

SEQ ID NO: 3 - protein, 710 aa, Campylobacter sputorum
MSNFNFAKFLNKLPRLSKHTILMIVLAVCFGIFCRFYWVVWASAYPHFIWNDELMISTNDGYAFAEGTRDMIAGFHQPNDLSYYGSSLSTLSMWLYSILPFSLETILLYMSTFLSPLLAVPLILIGKELNASKAGFIAALLAVVANSYYNRTMSGYYDTDMLNITLPMMVFWSITRLVQRKERVNLIFIPVFMAIYGWWYPSSYSLLLAMIGMFVLYTIVFERYEKLNYEAMVFMILAITSFPIQIKFIIVIILYALIYFYQRFFDKKVIFALIIASSICFIWLGGLNPILFNIKFYIFRDIADSGDTVFKFFNVNQTIRESSAIDFNTVATRISGHLIVFLVSIVGYILFIKNNKILLLTLPILFLGLMSFKSGLRFTIYSVPVMALGFGYFVMYCFTKIDIKDRFLGYAFLFVVTFSALYPSLKHIYDYKVFPVFTHSEVESLDDLKNIAKREDYVLSWWDYGYPIRYYSDVKTLIDGGKHLGSDNFAVSFALGSDQNSSANMARLEVEYTERNYEEKFGLNLKQIMKDYNATNVNEFLLSLKDANLALPKQTRDIYYYLPDRMIYIYPTVLAFSRLDLTTGQEFAEPFFIVSERFSATNDNQIMLNNNVILSSDGTKLSINGNSYSVNTYVETSYDQNEKLNVNYFNIDPNSNFYVIFMKDYLRILVLDKTLYDSAYIQLFVLENYDKNLFEPVILNGSTKIYKLKK

SEQ ID NO: 4 - DNA, 840 bp, Pseudomonas aeruginosa
atgaaaaaaatacttctaagtgttttaacggcctttgttgcagtagtattggctgcttgtggaggaaattctgactctaaaactttaaattctcttgataagatcaagcaaaatggagttgttaggattggggtatttggcgataaaccaccttttggttatgtggatgaaaaaggaaacaatcaaggctatgatatagctttagctaaacgcatagcaaaagaactttttggcgatgaaaataaggtgcaatttgttcttgttgaagctgcaaatagggttgagtttttaaaatcaaataaagtagatattattttggctaattttactcaaactccgcaaagggcagagcaggttgatttttgctcgccttatatgaaggtagctttaggcgtagctgtaccaaaggatagtaatataactagcgtagaagatttaaaagataaaaccttgcttttaaacaaaggcacaacagcagatgcttattttacgcaaaattatcctaatattaaaactttaaaatatgatcaaaataccgaaacctttgccgctttgatggataaaagaggcgatgctttaagtcatgataataccttactttttgcttgggtgaaagatcatcctgattttaaaatgggtattaaagagttaggtaacaaagatgttatcgcaccagcggttaaaaaaggcgataaagaacttaaagaatttatcgataatttgatcatcaaactaggccaagagcagttttttcacaaggcttatgatgaaactttaaaagctcattttggagatgatgttaaggccgatgatgtagtgattgaaggtggaaaaatttaa

SEQ ID NO: 5 - protein, 279 aa, Pseudomonas aeruginosa
MKKILLSVLTAFVAVVLAACGGNSDSKTLNSLDKIKQNGVVRIGVFGDKPPFGYVDEKGNNQGYDIALAKRIAKELFGDENKVQFVLVEAANRVEFLKSNKVDIILANFTQTPQRAEQVDFCSPYMKVALGVAVPKDSNITSVEDLKDKTLLLNKGTTADAYFTQNYPNIKTLKYDQNTETFAALMDKRGDALSHDNTLLFAWVKDHPDFKMGIKELGNKDVIAPAVKKGDKELKEFIDNLIIKLGQEQFFHKAYDETLKAHFGDDVKADDVVIEGGKI

SEQ ID NO: 6 - DNA, 1104 bp, Campylobacter jejuni
atgaaattatttcaaaaaaatactattttagctttaggtgttgtgcttttactcactgcttgcagcaaagaagaagcaccaaaaatacaaatgccgcctcaacctgtaacaaccatgagtgctaaatctgaagatttaccacttagttttacttaccctgctaaacttgtcagtgattatgatgtcattataaagcctcaagttagtggcgtaatagaaaataaactttttaaagctggagataaagtaaaaaaaggacaaacattatttattatagaacaagacaaatttaaagctagtgttgattcggcttacggacaagctttgatggctaaggcaactttcgaaaatgcaagcaaggattttaatcgttctaaagctctttttagtaaaagtgcaatctctcaaaaggaatacgactcttctcttgctacatttaacaattcaaaagctagtctagcaagtgctagagcacagcttgcaaatgcaagaattgatctagatcataccgaaataaaagctccttttgatggtactataggagatgctttagttaatataggagattatgtaagtgcttcaacaactgaactagttagagttacaaatttaaatcctatttacgcagatttctttatttcagatacagataaactaaatttagtccgcaatactcaaaatggaaaatgggatttagacagcattcatgcaaatttaaatcttaatggagaaaccgttcaaggcaaactttattttattgattctgttatagatgctaatagtggaacagtaaaagccaaagctatatttgacaacaacaactcaacacttttaccaggtgcttttgcaacaattacttcagaaggttttatacaaaaaaatggctttaaagtgcctcaaatagctgttaaacaaaatcaaaatgatgtttatgttcttcttgttaaaaatggaaaagtagaaaaatcttctgtacatataagctaccaaaacaatgaatatgccattattgacaaaggattacaaaatggcgataaaatcattttagataactttaaaaaaattcaagttggtagcgaagttaaagaaattggagcacaataa

SEQ ID NO: 7 - protein, 367 aa, Campylobacter jejuni
MKLFQKNTILALGVVLLLTACSKEEAPKIQMPPQPVTTMSAKSEDLPLSFTYPAKLVSDYDVIIKPQVSGVIENKLFKAGDKVKKGQTLFIIEQDKFKASVDSAYGQALMAKATFENASKDFNRSKALFSKSAISQKEYDSSLATFNNSKASLASARAQLANARIDLDHTEIKAPFDGTIGDALVNIGDYVSASTTELVRVTNLNPIYADFFISDTDKLNLVRNTQNGKWDLDSIHANLNLNGETVQGKLYFIDSVIDANSGTVKAKAIFDNNNSTLLPGAFATITSEGFIQKNGFKVPQIAVKQNQNDVYVLLVKNGKVEKSSVHISYQNNEYAIIDKGLQNGDKIILDNFKKIQVGSEVKEIGAQ

SEQ ID NO: 8 - DNA, 2112 bp, Pseudomonas aeruginosa
atgaaaaagatttggctggcgctggctggtttagttttagcgtttagcgctagcgatcagaacgcgaccggcggtgaccaaaatgccacaggtggcgatcaaaacgccaccggcggtgaccagaatgcgacagccgccgaggaagccttcgacctctggaacgaatgcgccaaggcctgcgtgctcgacctcaaggacggcgtgcgttccagccgcatgagcgtcgacccggccatcgccgacaccaacggccagggcgtgctgcactactccatggtcctggagggcggcaacgacgcgctcaagctggccatcgacaacgccctcagcatcaccagcgacggcctgaccatccgcctcgaaggcggcgtcgagccgaacaagccggtgcgctacagctacacgcgccaggcgcgcggcagttggtcgctgaactggctggtaccgatcggccacgagaagccctcgaacatcaaggtgttcatccacgaactgaacgccggtaaccagctcagccacatgtcgccgatctacaccatcgagatgggcgacgagttgctggcgaagctggcgcgcgatgccaccttcttcgtcagggcgcacgagagcaacgagatgcagccgacgctcgccatcagccatgccggggtcagcgtggtcatggctcaggcccagccgcgccgggaaaagcgctggagcgaatgggccagcggcaaggtgttgtgcctgctcgacccgctggacggggtctacaactacctcgcccagcagcgctgcaacctcgacgatacctgggaaggcaagatctaccgggtgctcgccggcaacccggcgaagcatgacctggacatcaaggataataataattctactcccacggtcatcagtcatcgcctgcatttccccgagggcggcagcctggccgcgctgaccgcgcaccaggcctgccacctgccgctggaggccttcactcgtcatcgccagccgcgcggctgggaacaactggagcagtgcggctatccggtgcagcggctggtcgccctctacctggcggcgcgactgtcgtggaaccaggtcgaccaggtgatccgcaacgccctggccagccccggcagcggcggcgacctgggcgaagcgatccgcgagcagccggagcaggcccgtctggccctgaccctggccgccgccgagagcgagcgcttcgtccggcagggcaccggcaacgacgaggccggcgcggccagcgccgacgtggtgagcctgacctgccccgtcgccaaagatcaaaatagaactaaaggggaatgcgcgggcccggcggacagcggcgacgccctgctggagcgcaactatcccactggcgcggagttcctcggcgacggcggcgacgtcagcttcagcacccgcggcacgcagaactggacggtggagcggctgctccaggcgcaccgccaactggaggagcgcggctatgtgttcgtcggctaccacggcaccttcctcgaagcggcgcaaagcatcgtcttcggcggggtgcgcgcgcgcagccaggacctcgacgcgatctggcgcggtttctatatcgccggcgatccggcgctggcctacggctacgcccaggaccaggaacccgacgcgcgcggccggatccgcaacggtgccctgctgcgggtctatgtgccgcgctggagtctgccgggcttctaccgcaccggcctgaccctggccgcgccggaggcggcgggcgaggtcgaacggctgatcggccatccgctgccgctgcgcctggacgccatcaccggccccgaggaggaaggcgggcgcgtgaccattctcggctggccgctggccgagcgcaccgtggtgattccctcggcgatccccaccgacccgcgcaacgtcggcggcgacctcgacccgtccagcatccccgacaaggaacaggcgatcagcgccctgccggactacgccagccagcccggcaaaccgccgcgcgaggacttgaaggatcagaacgcgaccggcggtgaccaaaatgccacaggtggcgatcaaaacgccaccggcggtgaccagaatgcgacagtcgaccatcaccatcatcaccattga

SEQ ID NO: 9 - protein, 697 aa, Pseudomonas aeruginosa
MKKIWLALAGLVLAFSASDQNATGGDQNATGGDQNATGGDQNATAAEEAFDLWNECAKACVLDLKDGVRSSRMSVDPAIADTNGQGVLHYSMVLEGGNDALKLAIDNALSITSDGLTIRLEGGVEPNKPVRYSYTRQARGSWSLNWLVPIGHEKPSNIKVFIHELNAGNQLSHMSPIYTIEMGDELLAKLARDATFFVRAHESNEMQPTLAISHAGVSVVMAQAQPRREKRWSEWASGKVLCLLDPLDGVYNYLAQQRCNLDDTWEGKIYRVLAGNPAKHDLDIKDNNNSTPTVISHRLHFPEGGSLAALTAHQACHLPLEAFTRHRQPRGWEQLEQCGYPVQRLVALYLAARLSWNQVDQVIRNALASPGSGGDLGEAIREQPEQARLALTLAAAESERFVRQGTGNDEAGAASADVVSLTCPVAKDQNRTKGECAGPADSGDALLERNYPTGAEFLGDGGDVSFSTRGTQNWTVERLLQAHRQLEERGYVFVGYHGTFLEAAQSIVFGGVRARSQDLDAIWRGFYIAGDPALAYGYAQDQEPDARGRIRNGALLRVYVPRWSLPGFYRTGLTLAAPEAAGEVERLIGHPLPLRLDAITGPEEEGGRVTILGWPLAERTVVIPSAIPTDPRNVGGDLDPSSIPDKEQAISALPDYASQPGKPPREDLKDQNATGGDQNATGGDQNATGGDQNATVD

SEQ ID NO: 10 - DNA, 14645 bp, Campylobacter jejuni
atgaaaattcttattagcggtggtgcaggttatataggttctcatactttaagacaatttttaaaaacagatcatgaaatttgtgttttagataatctttctaagggttctaaaatcgcaatagaagatttgcaaaaaacaagagcttttaaatttttcgaacaagatttaagtgattttcaaggcgtaaaagcattgtttgagagagaaaaatttgacgctattgtgcattttgcagcaagcattgaagtttttgaaagtatgcaaaatcctttaaaatattatatgaacaacactgttaatacgacaaatctcatcgaaacttgtttgcaaactggagtgaataaatttatattttcttcaacggcggccacttatggcgaaccacaaactcccgttgtgagcgaaacaagtcctttagcacctattaatccttatgggcgtagtaagcttatgagtgaagaagttttgcgtgatgcaagtatggcaaatcctgaatttaagcattgtattttaagatattttaatgttgcaggtgcttgtatggattatactttaggacaacgctatccaaaagcgactttgcttataaaagttgcagctgaatgtgccgcaggaaaacgtgataaacttttcatatttggcgatgattatgatacaaaagatggtacttgcataagagattttatccatgtagatgatatttcaagtgcacatttagcggctttggattatttaaaagagaatgaaagcaatgtttttaatgtaggttatggacatggttttagcgtaaaagaagtgattgaagcgatgaaaaaagttagcggagtggattttaaagtagaacttgccccacgccgtgcgggtgatcctagtgtattgatttctgatgcaagtaaaatcagaaatcttacttcttggcagcctaaatatgatgatttagagcttatttgtaaatctgcttttgattgggaaaaacagtgttaaaaaaacttttttttattttaagcaaggaagataaaaattttttatttttcttgcttgttttttcagtatttgtttcttttatagaaacttttgcgatttctttggtaatgccttttatcactttggctagtgatttttcttattttgatcgtaataaatatttaatcagcctaaaagaatatcttaatatccctgtttttgaaatcattgtttattttggagtggggcttattgttttttatgtatttagagctttgttaaatgcgtattattttcatcttttggcaagattttctaaaggacgttatcatgcgatcgcttataaggttttttctaaatttttaaatattaattatgaaaaatttactcaaaaaaatcaatctgaaattttaaagtccattacaggggaagtttataatctaagcactatgatttcatcatttttacttttgatgagtgaaatttttgtagtgcttttgctttatgctttaatgcttttgattaattataaaatcactttatttttaagtatttttatggtgttaaatgcttttattttagtgaaaattttaagccctatcattaaaaaagcaggactaagacgcgaagaagcgatgaaaaatttcttcgaaattttaaatacaaatttaaataattttaaatttatcaagcttaaaaccaaagaagatggagtattaagtctttttaaagcacaaagtgaagctttttctaaagcaaatattaccaatgaaagcgtagctgcggtgcctagaatttatcttgaaggaataggcttttgtgtgcttgtttttatcgtggtatttttggttttgaaaaatgaaagtgatatttcaggtattttatccacgatttctatttttgttttagcgctttatcgcttaatgccaagcgcaaatcgtattatcacaagttatcatgatttgctttattatcattcttctttgaatattatttatcaaaatttaagacaagaagaagaaaatttgggcgagggaaaattaagttttaatcaagagcttaaaatttgcaatcttagctttggttatgagggaaaaaaatatttatttaaaaatcttaatttaaacattaaaaaaggtgaaaaaatcgcttttataggggagagtggttgtggaaaaagtaccttagtagatcttatcataggacttttaaaaccaaaagaagggcaaattttaattgataagcaagaattaaatgcaagtaatgcaaaaaattatcgccaaaaaataggctatatcccgcaaaatatctatctttttaatgatagcatagctaaaaatatcacttttggagatgcggttgatgaagaaaaacttaataaggttatcaaacaagcaaatttagagcattttataaaaaatttacctcaaggagttcagacaaaagtaggcgatggggggagtaatttaagcgggggacaaaaacaacgcatagctatagcaagggctttgtatttagagcctgaaattttagtgcttgatgaagcaacttctgcgcttgatactcaaagtgaagcaaaaatcatggatgaaatttataaaatttctaaagataaaaccatgattattatcgcacatcgcctttctacgataacgcaatgtgataaggtttatcgtttagaacacggtaagcttaaagaggagaaatgatgaaaataagctttattatcgcaactttaaattcaggaggcgctgagcgtgttttagtaaccttagctaatgcgctttgcaaagagcatgaagtaagtattattaaatttcatacaggagaatctttttataagcttgaaaatgaagttaaagttacaagtttagaacaatttagatttgacacgctttatcataaaatcgcaagtcgttttaagaaattttttgccttaagaaaggctttaaaagaaagtaaggctgatgtttttatttcttttttggatacaactaatattgcttgtattctagctaatataggacttaaaactccactcatcattagcgagcatagtaatgaagcgtatttaaaacctaaaacttggcgttttttaagaagggtaagctatcctttttgtgatgctttaagtgtgcttggaagcagtgataaggtgtattatgaaagatttgtaaaaagggttaagcttttattaaacccttgtcattttagcgatgaaattccttttgattctagttttgaaaaagaaaatttggttctttttatagggcgtttagatcacaacaaaaaccctgtaatgtttttaaaagctatagcacatttggataaaaatttgcaagaaaattataaatttgttatagcaggagatggagagttaaggcaagaacttgaatacaaggtaaaatctttaggaataaaagttgattttttaggacgcgttgaaaatgtcaaggctctttatgaaaaagcaaaagtgctttgcctttgttcttttgtagagggtttgccaacggttttaattgaaagtttgtattttgaggtttgtagaatttcaagttcttattataatggtgctaaggatttaatcaaagataatcatgatgggcttttggtaggttgtgatgatgaaatagcacttgctaaaaaacttgaacttgttttaaatgatgaaaattttagaaaagaacttgtaaataatgccaaacaaaggtgtaaagactttgaaatttctaacatcaaagaagaatggcttaagcttatagtcgaggttaaaaatgcctaaactttctgttatagtgccaacttttaatcgtcaagttttgttagaaaaggctattaaaagcatacaaaatcaagattttaaagatttagaaatcattgtaagcgatgataattctagtgatgatactaaaagtgtggtgcaaaatttacaaaaagatgatgatcgcattaagtattttttaaatcaaaattacaaacaaggcccaaatggcaataaaaacaatggcttagatcaagcaagtggcgagtttgtaacttttttagatgatgatgatgagcttttatctggggctttaagtaccttgatgcaaaaagcaaatgagggttatgctcatgtttttggaaattgtttgatagaaaaagaaggaaatttaagcaaggaatttagcggtaagggcttggaaaaagatagtgaaatttctaaaaaagattttttaatggctaaatttagcggagagtttttttctgtttttaaaaaatctctacttgaaaacaagcgttttaatgaagaattttatggcaatgaagccacgctttgggtaaatttatacaaggaaaaaagtttttatatccataaggcttttaggatttataggatttttaggcaagatagcgtgactttaggggcgagtaaaaatgctcatagggtgtatttgggatatttagagcttgctaaaattttagaaaatgaacttagaatgagtaaggataaagattataaaaaaacttgtgcgagttattataaaatggcagcttattatgcaaaacttgcaaaaaattataaagctctttataagtgtttgtttaaaagcctgagtataaaaatcaacgctcctgctttgatattactcattttaagtataattccaaataatatgattgaaaaattatcaaaaattcgggtggctttatgcaaaaattaggcatttttatttattctttaggaagtggtggtgctgaaagagttgtggcgactttattgcctattttaagtttgaaatttgaagtgcatttgattttaatgaatgataaaatttcttatgaaattccagagtgtcaaattcattttttagaatgttcaaaacctagtgaaaatcctattttgaaatttttaaaactaccttttttggctttaaaatataaaaaactttgcagaaatttaggcattgatacagaatttgtttttttaaatcgacctaattatatagccttaatggcaagaatgtttggaaacaaaactcgccttgtgatcaatgaatgcactacgccaagtgtgatgtatgcgaaaaataattttaattctttggcaaataaatttttaatttctttgctttacccaaaagctgatttaatcttgcctaattctaagggaaatttagaagatttagtgcaaaattttagtataaatccaaaaaaatgtgaaattttatacaatgccatcgatttagaaaatatagagcaaaaagctcttgaagatgtagctttaaaagataaatttattttaagtgtaggcaggcttgataaaggtaaaaatcatgctttattaattcgtgcttatgcaagattgaaaacagatttaaagcttgtgattttaggtgaaggtgtgcttaaagatgagcttttagctttgattaaagagttaaatttagaagaaaaggttttgcttttaggatttgataataatccttataaatacatggctaaatgcgaattttttgcttttgcttctgtatttgaaggcttttcaaatgttttaattgaaagcttagcttgttcttgtgcggtggtttgcactgatcataaaagtggcgcaagagagctttttggcgatgatgaatttggacttttagtagaagtagataatgaaaactccatgtttcagggtttaaagactatgcttgaagacgataaattaagaaaagcgtataaaaataaggctaaaactagggctaaagcttttgataaagtaaaaattgcacgcgatgctttgaaatatttattaggataaaagatgttgaaaaaagagtatttaaaaaacccttatttagttttgtttgcgatgattatattagcttatgtttttagtgtattttgcaggttttattgggtttggtgggcaagtgagtttaatgagtattttttcaataatcagttaatgatcatttcaaatgatggctatgcttttgctgagggcgcaagagatatgatagcaggttttcatcagcctaatgatttgagttattatggatcttctttatccgcgcttacttattggctttataaaatcacacctttttcttttgaaagtatcattttatatatgagtacttttttatcttctttggtggtgattcctactattttgctagctaacgaatacaaacgtcctttaatgggctttgtagctgctcttttagcaagtatagcaaacagttattataatcgcactatgagtgggtattatgatacggatatgctggtaattgttttgcctatgtttattttattttttatggtaagaatgattttaaaaaaagactttttttcattgattgccttgccgttatttataggaatttatctttggtggtatccttcaagttatactttaaatgtagctttaattggactttttttaatttatacacttatttttcatagaaaagaaaagattttttatatagctgtgattttgtcttctcttactctttcaaatatagcatggttttatcaaagtgccattatagtaatactttttgctttattcgccttagagcaaaaacgcttaaattttatgattataggaattttaggtagtgcaactttgatatttttgattttaagtggtggggttgatcctatactttatcagcttaaattttatatttttagaagtgatgaaagtgcgaatttaacgcagggctttatgtattttaatgtcaatcaaaccatacaagaagttgaaaatgtagatcttagcgaatttatgcgaagaattagtggtagtgaaattgtttttttgttttctttgtttggttttgtatggcttttgagaaaacataaaagtatgattatggctttacctatattggtgcttgggtttttagccttaaaaggggggcttagatttaccatttattctgtacctgtaatggccttaggatttggttttttattgagcgagtttaaggctataatggttaaaaaatatagccaattaacttcaaatgtttgtattgtttttgcaactattttgactttagctccagtatttatccatatttacaactataaagcgccaacagttttttctcaaaatgaagcatcattattaaatcaattaaaaaatatagccaatagagaagattatgtggtaacttggtgggattatggttatcctgtgcgttattatagcgatgtgaaaactttagtagatggtggaaagcatttaggtaaggataattttttcccttcttttgctttaagcaaagatgaacaagctgcagctaatatggcaagacttagtgtagaatatacagaaaaaagcttttatgctccgcaaaatgatattttaaaaacagacattttgcaagccatgatgaaagattataatcaaagcaatgtggatttgtttctagcttcattatcaaaacctgattttaaaatcgatacgccaaaaactcgtgatatttatctttatatgcccgctagaatgtctttgattttttctacggtggctagtttttcttttattaatttagatacaggagttttggataaaccttttacctttagcacagcttatccacttgatgttaaaaatggagaaatttatcttagcaacggagtggttttaagcgatgattttagaagttttaaaataggtgataatgtggtttctgtaaatagtatcgtagagattaattctattaaacaaggtgaatacaaaatcactccaattgatgataaggctcagttttatattttttatttaaaggatagtgctattccttacgcacaatttattttaatggataaaaccatgtttaatagtgcttatgtgcaaatgttttttttaggaaattatgataagaatttatttgacttggtgattaattctagagatgctaaggtttttaaacttaaaatttaagggttgaaaatgagaataggatttttatcacatgcaggagcaagtatttatcattttagaatgcctattataaaagcattaaaagatagaaaagatgaagtttttgttatagtgccgcaagatgaatacacgcaaaaacttagagatcttggtttaaaagtaattgtttatgagttttcaagagctagtttaaatccttttgtagttttaaagaattttttttatcttgctaaggttttaaaaaatttaaatcttgatcttattcaaagtgcggcacacaaaagcaatacctttggaattttagcggcaaaatgggcaaaaattccttatcgttttgctttggtagaaggcttgggatctttttatatagatcaaggttttaaggcaaatttagtacgttttgttattaataatctttataaattaagttttaaatttgcacaccaatttatttttgtcaatgaaagtaatgccgagtttatgcggaatttaggacttaaggaaaataaaatttgtgtgataaaatccgtagggatcaatttaaaaaaattttttcctatttatatagaatcggaaaaaaaagagcttttttggagaaatttaaatatagataaaaaacctattgttcttatgatagcaagagctttatggcataaaggtgtaaaagaattttatgaaagtgctactatgctaaaagacaaagcaaattttgttttagttggtggaagagatgaaaatccttcttgtgcgagtttggagtttttaaactcgggtgtggtgcattatttgggtgctagaagtgatatagtcgagcttttgcaaaattgtgatatttttgttttaccaagctataaagaaggctttcctgtaagtgttttggaggcaaaagcttgtggcaaggctatagtggtgagtgattgtgaaggttgtgtagaggctatttctaatgcttatgatggactttgggcaaaaacaaaaaatgctaaggatttaagcgaaaaaatttcacttttattagaagatgaaaaattaagattaaatttagctaaaaatgctgcccaagatgctttacaatacgatgaaaataatatcgcacagcgttatttaaaactttatgatagggtaattaagaatgtatgaaaaagtttttaaaagaatttttgattttattttagctttagtgcttttagtacttttttctccggtgattttaatcactgctttacttttaaaaatcactcaaggaagtgtgattttcactcaaaatcgccctgggttagatgaaaaaatttttaaaatttataaatttaaaaccatgagcgatgaaagagatgagaagggtgagttattaagcgatgaattgcgtttgaaagcctttggaaaaattgttagaagcttaagtttggatgagcttttgcaactttttaatgttttaaaaggggatatgagttttgtggggcctagacctcttttggttgagtatttatccctttataatgaagagcaaaaattgcgccataaggtgcgtccaggtataacaggatgggcgcaggtaaatggcagaaatgctatttcttggcagaaaaaattcgaacttgatgtgtattatgtgaaaaatatttcttttttgcttgatttaaaaatcatgtttttaacagctttaaaggttttaaaacgaagcggggtaagcaaagaaggccatgttacaacagagaaatttaatggcaagaactgaaaaaatttatatttatggtgctagtggtcatgggcttgtttgtgaagatgtggctaaaaatatgggctataaagaatgtatttttttagatgattttaaaggaatgaaatttgaaaacaccttgcctaaatatgatttttttatagctataggaaacaatgaaattcgaaaaaagatttatcaaaaaatttcagaaaatggctttaaaatagttaatcttattcataaaagtgcacttataagtcctagtgcaagcgtggaagaaaatgcagggattttaattatgccctatgtagtgattaacgctaaagccaaaatagaaaaaggcgtgattttaaatacttcaagtgtgattgagcatgaatgcgtgataggggaattttctcatgtaagcgtaggggctaaatgtgcgggtaatgtaaaaatcggtaaaaattgttttttagggattaattcttgtgttttgcctaatttaagcttagcagatgatagtattttgggtggtggagcaactttggttaaaagccaaaatgaaaaaggtgtttttgtgggagtgcctgcaaaaagaaaaatatgaaatgattataaaaagatttttgtttgattctttgtaaatttttttaggtaaaatagagttaatttataaaaattttgttttatacaaaggataaatcatgagattttttctttctcctccgcatatgggcggtaatgaattaaaatatatagaagaagttttcaaaagcaattatatagcacctttgggtgaatttgtaaatcgctttgagcaaagtgtaaaagattatagcaaaagtgaaaatgccttagctttaaattcagctacagcagctttgcatttagctttaagggtggcaggggtaaaacaagatgatattgttttggcttcttcttttacttttatcgcttcagtggcgcctatttgttatcttaaagcaaaacctgtatttatagattgtgatgaaacttataatatcgatgtagatttgttaaaacttgctattaaggaatgtgaaaaaaaaccaaaagcattgattttaactcatctttatggcaatgcggctaaaatggatgaaattgttgaaatttgcaaggaaaatgaaattgttttaatcgaagatgctgctgaagctttaggaagtttttataagaataaagccttaggaacttttggagaatttggagcttattcttataatggcaataaaattatcaccacttcaggtggaggtatgcttataggaaaaaataaagaaaagattgaaaaagcaagattttatagcactcaagctagggaaaattgtttgcattatgaacatttagactatggttataattaccgtttaagcaatgttttaggagctattggtgtagcacaaatggaggttttagaacaaagagtgcttaaaaaaagagaaatttatgagtggtataaagaatttttaggagagtattttagctttttagatgaattagaaaattcaagaagtaatcgctggttaagtacagctttgattgattttgataaaaatgaacttaatgcttgtcaaaaagatataaatatcagtcaaaaaaatattactttgcatccaaaaatttcaaaactcatagaagatttgaaaaatgaacaaatagaaacaagaccattatggaaagctatgcacactcaagaagtatttaaaggaactaaggcttatcttaatggcaatagtgagttatttttccaaaaaggaatttgtttgccaagtggtacggcgatgagcaaagatgatgtttatgaaatttcaaaactgatcttaaagagcataaaggcttaaaatgattttttataaaagcaaaagattagcattttttttaacttcagatattgttttaattttacttagtgtttatctggctttttctttgagatttagtggagatattccgagtattttttatcatggcatgatggtttctgctattattttgcttgttttaaaactttcatttttgtttgtttttagaatttataaagtagcttggagatttttttccctcaatgaagcaagaaaaatttttatcgctttgcttttagctgagttttgtttttttcttattttttatttttttagtgatttttttaatccttttccaagaagtgctattgtgatagattttgttctttcttatatgtttataggtactttaagaattagcaaaagaatgcttgtggattttaaaccttctaaaatgaaagaagaagaaactccttgtattgtagtaggggcaacttctaaggctttacatttgttaaaaggcgcaaaagaaggttctttagggctttttcctgtgggcgtagttgatgcgagaaaagagcttatagggacttattgtgataaatttgttgtagaagaaaaagaaaaaataaaatcttatgtagaacaaggggtaaaaactgccattattgctttaagacttgaacaagaagagcttaaaaaactttttgaagaacttgtagcttatggtatttgtgatgtaaaaatattttcttttacaagaaatgaagcaagagatattagtatagaagacttgcttgctagaaaaccaaaagatttagacgatagtgctgtggcggcttttttaaaagacaaggtagttttggtaagtggagcaggtggaactataggcagtgaactttgtaagcaatgtattaaatttggtgctaagcatcttattatggttgatcatagtgagtataatctttataagatcaatgatgatttaaatttatataaagaaaaaattactcctattttgttaagtattttagataagcaaagtttagatgaggtattaaaaacttataaacctgagcttattttacatgcagccgcttataaacatgtgcctctttgcgaacaaaatccacattcagcagtaatcaataatattttaggaaccaaaattttatgcgacagtgctaaagaaaataaagtagctaaatttgtgatgataagtacagataaagcagtacgaccaacaaatattatgggttgcactaagagagtttgtgagctttatactttaagtatgagtgatgaaaattttgaagttgcttgtgtgcgttttggtaatgttttaggttctagtggtagtgtgataccgaaatttaaagcacaaattgccaataatgagcctttaactttaacacaccctgatatagtgcgttattttatgcttgtggctgaggcagtgcaacttgttttgcaagctggagctatcgcaaaagggggagaactttttgttttggatatgggtaagcctgtgaaaatcatagatttagctaaaaaaatgcttttactttctaatcgcaatgatttagaaattaaaatcacaggtttaagaaaaggtgagaagctttatgaagagcttttgattgatgaaaatgatgctaaaacccaatatgagagtatttttgtagcaaagaatgagaaggttgatcttgattggcttaataaagagatagaaaatttacaaatatgtgaagatatttcagaggctttattaaagattgtacctgaatttaaacacaataaagaaggcatataatgtatataaaagatatacaaagatttgaagataatcgctatcgtgctagagcttatatgagttatattttaacaagaaatctacccaataaacttcctgatattcaccttgaaacgattaaaacagctttggataaaatagctcatgaagttgttgtttttgatgctttgtatattttagatatttcaggcatgcaaatagaaaatgcgatttccttaaataaggctcatgaaatagggcagggtgaggatagaagtactcgttcttatttttatagagctgtaaaattaaaacgatgtgttttgagcgatccttatccttcggttttaaacaatgaactttgcgtaacagcttctataccaatttacgatgataaaaataacttgctttttgttgtttgtattgatatcaagcttgaagatattttaaagattattcaagcaggaaaatttgagtttgtttttactcaatttagtcgtttggtgtatttttgtttcgcactggttttatttgtgattacttgttttttatttcaaaaaggtttttttagtctttttgataatcaagctataggcatagaacatatgtttgaaagtaccattgccataactttagctttagctatttttgatttggcaaaaactttgatcgaacaagaagtattaggaaggacaaaaaaagaagaaggtggaattcaaaaaaccatggtgagatttttgggttctattatcattgctttagctatagaagctttgatgttggtatttaaacttgctattggtgatctttctcagatgatttatgcgatttatcttatcggtggagtgagcttgcttcttttaggcttaagtgtatatttatttacggttaagtataaaaataataatatttgagtaaaaatttaagtaaaagatgatataatgctgttttttaaaattttttagcttgattaataaggctaaaaagggtaaaataaaactataaaaactttgaaaggacgaaattgtgaaattgttagttgttgatgacagttctactatgagaaggattattaaaaataccctaacaagacttggacacgatgatgttttagaagctgagcatggcgttgaagcttgggatttattaactaaaaatgaagatgtaaaagttttaattacagattggaatatgccagaaatgaatggcttggagttggtaaaaaaagtaagagcagagaaaaaatatgaagatatgcctattatcatggttacaactgagggcggaaaagctgaagtgattactgctttaaaagctggcgtaaataactatattgtaaaaccttttactccacaagttttaaaggaaaaacttgaagatgttttaggaacaggaagtggagaaggtgcagctgagtaa

SEQ ID NO: 11 - DNA, 31 bp, artificial sequence
  primer
ttttgcggccgcttctacgtgttccgcttcc

SEQ ID NO: 12 - DNA, 31 bp, artificial sequence
  primer
ttttgcggccgcattgcgttgcgctcactgc

SEQ ID NO: 13 - DNA, 603 bp, artificial sequence
  transposon
ggccgcctaggccgcggccgcctacttcgtatagcatacattatacgaagttatgtctgacgctcagtggaacgacgcgtaactcacgttaagggattttggtcatgatcagcacgttgacaattaatcatcggcatagtatatcggcatagtataatacgacaaggtgaggaactaaaacatggccaagttgaccagtgccgttccggtgctcaccgcgcgcgacgtcgccggagcggtcgagttctggaccgaccggctcgggttctcccgggacttcgtggaggacgacttcgccggtgtggtccgggacgacgtgaccctgttcatcagcgcggtccaggaccaggtggtgccggacaacaccctggcctgggtgtgggtgcgcggcctggacgagctgtacgccgagtggtcggaggtcgtgtccacgaacttccgggacgcctccgggccggccatgaccgagatcggcgagcagccgtgggggcgggagttcgccctgcgcgacccggccggcaactgcgtgcacttcgtggccgaggagcaggactgaataacttcgtatagcatacattatacgaagttatggccgcctaggcc

SEQ ID NO: 14 - DNA, 19 bp, artificial sequence
  primer
gcgctggctggtttagttt

SEQ ID NO: 15 - DNA, 18 bp, artificial sequence
  primer
cgcattcgttccagaggt

SEQ ID NO: 16 - DNA, 20 bp, artificial sequence
  primer
gacaaggaacaggcgatcag

SEQ ID NO: 17 - DNA, 20 bp, artificial sequence
  primer
tggtgatgatggtgatggtc

SEQ ID NO: 18 - DNA, 2142 bp, Campylobacter jejuni
atgttgaaaaaagagtatttaaaaaacccttatttagttttgtttgcgatgattgtattagcttatgtttttagtgtattttgcaggttttattgggtttggtgggcaagtgagtttaacgagtattttttcaataatcaattaatgatcatttcaaacgatggctatgcttttgctgagggcgcaagagatatgatagcaggttttcatcagcctaatgatttgagttattatggatcttctttatctacgcttacttattggctttataaaatcacacctttttcttttgaaagtatcattttatatatgagtacttttttatcttctttggtggtgattcctattattttactagctaatgaatacaaacgccctttaatgggctttgtagctgctcttttagcaagtgtagcaaacagttattataatcgcactatgagtgggtattatgatacggatatgctggtaattgttttacctatgtttattttattttttatggtaagaatgattttaaaaaaagactttttttcattgattgccttgccattatttataggaatttatctttggtggtatccttcaagttatactttaaatgtagctttaattggactttttttaatttatacacttatttttcatagaaaagaaaagattttttatatagctgtgattttgtcttctcttactctttcaaatatagcatggttttatcaaagtgccattatagtaatactttttgctttatttgctttagagcaaaaacgcttaaattttatgattataggaattttaggtagtgcaactttgatatttttgattttaagtggtggggttgatcccatactttatcagcttaaattttatatttttagaagcgatgaaagtgcgaatttaacacagggctttatgtattttaatgttaatcaaaccatacaagaagttgaaaatgtagattttagcgaatttatgcgaagaattagtggtagtgaaattgttttcttgttttctttgtttggttttgtatggcttttgagaaaacataaaagtatgattatggctttacctatattggtgcttgggtttttagccttaaaaggaggacttagatttaccatttattctgtacctgtaatggctttaggatttggttttttattgagcgagtttaaggctatattggttaaaaaatatagccaattaacttcaaatgtttgtattgtttttgcaactattttgactttggctccagtatttatccatatttacaactataaagcgccaacagttttttctcaaaatgaagcatcattattaaatcaattaaaaaatatagccaatagagaagattatgtggtaacttggtgggattatggttatcctgtgcgttattatagcgatgtgaaaactttagtagatggtggaaagcatttaggtaaggataattttttcccttctttttctttaagtaaagatgaacaagctgcagctaatatggcaagacttagtgtagaatatacagaaaaaagcttttatgctccgcaaaatgatattttaaaatcagacattttacaagccatgatgaaagattataatcaaagcaatgtggatttatttctagcttcattatcaaaacctgattttaaaatcgatacaccaaaaactcgtgatatttatctttatatgcccgctagaatgtctttgattttttctacggtggctagtttttcttttattaatttagatacaggagttttggataaaccttttacctttagcacagcttatccacttgatgttaaaaatggagaaatttatcttagcaacggagtggttttaagcgatgattttagaagttttaaaataggtgataatgtggtttctgtaaatagtatcgtagagattaattctattaaacaaggtgaatacaaaatcactccaatcgatgataaggctcagttttatattttttatttaaaggatagtgctattccttacgcacaatttattttaatggataaaaccatgtttaatagtgcttatgtgcaaatgttttttttgggaaattatgataagaatttatttgacttggtgattaattctagagatgctaaagtttttaaacttaaaatttaa

SEQ ID NO: 19 - protein, 5 aa, artificial sequence
  glycosylation motif
DVNVT

SEQ ID NO: 20 - protein, 5 aa, artificial sequence
  glycosylation motif
EVNAT

SEQ ID NO: 21 - protein, 5 aa, artificial sequence
  glycosylation motif
DQNAT

SEQ ID NO: 22 - protein, 5 aa, artificial sequence
  glycosylation motif
DNNNT

SEQ ID NO: 23 - protein, 5 aa, artificial sequence
  glycosylation motif
DNNNS

SEQ ID NO: 24 - protein, 5 aa, artificial sequence
  glycosylation motif
DQNRT

SEQ ID NO: 25 - protein, 5 aa, artificial sequence
  glycosylation motif
ENNFT

SEQ ID NO: 26 - protein, 5 aa, artificial sequence
  glycosylation motif
DSNST

SEQ ID NO: 27 - protein, 5 aa, artificial sequence
  glycosylation motif
DQNIS

SEQ ID NO: 28 - protein, 5 aa, artificial sequence
  glycosylation motif
DQNVS

SEQ ID NO: 29 - protein, 5 aa, artificial sequence
  glycosylation motif
DNNVS

SEQ ID NO: 30 - protein, 5 aa, artificial sequence
  glycosylation motif
DYNVS

SEQ ID NO: 31 - protein, 5 aa, artificial sequence
  glycosylation motif
DFNVS

SEQ ID NO: 32 - protein, 5 aa, artificial sequence
  glycosylation motif
DFNAS

SEQ ID NO: 33 - protein, 5 aa, artificial sequence
  glycosylation motif
DFNSS

SEQ ID NO: 34 - protein, 5 aa, artificial sequence
  glycosylation motif
DVNAT

SEQ ID NO: 35 - protein, 5 aa, artificial sequence
  glycosylation motif
DFNVT

SEQ ID NO: 36 - protein, 5 aa, artificial sequence
  glycosylation motif
DVNAS

SEQ ID NO: 37 - DNA, 37 bp, artificial sequence
  primer
aagaattcatgttgaaaaaagagtatttaaaaaaccc

SEQ ID NO: 38 - DNA, 62 bp, artificial sequence
  primer
aaccatggttaagcgtaatctggaacatcgtatgggtaaattttaagtttaaaaaccttagc

SEQ ID NO: 39 - DNA, 47 bp, Artificial Sequence
  primer
ttttgaattcgattatcgccatggcgtcaaattttaatttcgctaaa

SEQ ID NO: 40 - DNA, 41 bp, Artificial Sequence
  primer
ttttgaattcttattttttgagtttataaattttagttgat

SEQ ID NO: 41 - DNA, 13659 bp, Campylobacter jejuni
ttactcagctgcaccttctccacttcctgttcctaaaacatcttcaagtttttcctttaaaacttgtggagtaaaaggttttacaatatagttatttacgccagcttttaaagcagtaatcacttcagcttttccgccctcagttgtaaccatgataataggcatatcttcatattttttctctgctcttactttttttaccaactccaagccattcatttctggcatattccaatctgtaattaaaacttttacatcttcatttttagttaataaatcccaagcttcaacgccatgctcagcttctaaaacatcatcgtgtccaagtcttgttagggtatttttaataatccttctcatagtagaactgtcatcaacaactaacaatttcacaatttcgtcctttcaaagtttttatagttttattttaccctttttagccttattaatcaagctaaaaaattttaaaaaacagcattatatcatcttttacttaaatttttactcaaatattattatttttatacttaaccgtaaataaatatacacttaagcctaaaagaagcaagctcactccaccgataagataaatcgcataaatcatctgagaaagatcaccaatagcaagtttaaataccaacatcaaagcttctatagctaaagcaatgataatagaacccaaaaatctcaccatggttttttgaattccaccttcttctttttttgtccttcctaatacttcttgttcgatcaaagtttttgccaaatcaaaaatagctaaagctaaagttatggcaatggtactttcaaacatatgttctatgcctatagcttgattatcaaaaagactaaaaaaacctttttgaaataaaaaacaagtaatcacaaataaaaccagtgcgaaacaaaaatacaccaaacgactaaattgagtaaaaacaaactcaaattttcctgcttgaataatctttaaaatatcttcaagcttgatatcaatacaaacaacaaaaagcaagttatttttatcatcgtaaattggtatagaagctgttacgcaaagttcattgtttaaaaccgaaggataaggatcgctcaaaacacatcgttttaattttacagctctataaaaataagaacgagtacttctatcctcaccctgccctatttcatgagccttatttaaggaaatcgcattttctatttgcatgcctgaaatatctaaaatatacaaagcatcaaaaacaacaacttcatgagctattttatccaaagctgttttaatcgtttcaaggtgaatatcaggaagtttattgggtagatttcttgttaaaatataactcatataagctctagcacgatagcgattatcttcaaatctttgtatatcttttatatacattatatgccttctttattgtgtttaaattcaggtacaatctttaataaagcctctgaaatatcttcacatatttgtaaattttctatctctttattaagccaatcaagatcaaccttctcattctttgctacaaaaatactctcatattgggttttagcatcattttcatcaatcaaaagctcttcataaagcttctcaccttttcttaaacctgtgattttaatttctaaatcattgcgattagaaagtaaaagcatttttttagctaaatctatgattttcacaggcttacccatatccaaaacaaaaagttctcccccttttgcgatagctccagcttgcaaaacaagttgcactgcctcagccacaagcataaaataacgcactatatcagggtgtgttaaagttaaaggctcattattggcaatttgtgctttaaatttcggtatcacactaccactagaacctaaaacattaccaaaacgcacacaagcaacttcaaaattttcatcactcatacttaaagtataaagctcacaaactctcttagtgcaacccataatatttgttggtcgtactgctttatctgtacttatcatcacaaatttagctactttattttctttagcactgtcgcataaaattttggttcctaaaatattattgattactgctgaatgtggattttgttcgcaaagaggcacatgtttataagcggctgcatgtaaaataagctcaggtttataagtttttaatacctcatctaaactttgcttatctaaaatacttaacaaaataggagtaattttttctttatataaatttaaatcatcattgatcttataaagattatactcactatgatcaaccataataagatgcttagcaccaaatttaatacattgcttacaaagttcactgcctatagttccacctgctccacttaccaaaactaccttgtcttttaaaaaagccgccacagcactatcgtctaaatcttttggttttctagcaagcaagtcttctatactaatatctcttgcttcatttcttgtaaaagaaaatatttttacatcacaaataccataagctacaagttcttcaaaaagttttttaagctcttcttgttcaagtcttaaagcaataatggcagtttttaccccttgttctacataagattttattttttctttttcttctacaacaaatttatcacaataagtccctataagctcttttctcgcatcaactacgcccacaggaaaaagccctaaagaaccttcttttgcgccttttaacaaatgtaaagccttagaagttgcccctactacaatacaaggagtttcttcttctttcattttagaaggtttaaaatccacaagcattcttttgctaattcttaaagtacctataaacatataagaaagaacaaaatctatcacaatagcacttcttggaaaaggattaaaaaaatcactaaaaaaataaaaaataagaaaaaaacaaaactcagctaaaagcaaagcgataaaaatttttcttgcttcattgagggaaaaaaatctccaagctactttataaattctaaaaacaaacaaaaatgaaagttttaaaacaagcaaaataatagcagaaaccatcatgccatgataaaaaatactcggaatatctccactaaatctcaaagaaaaagccagataaacactaagtaaaattaaaacaatatctgaagttaaaaaaaatgctaatcttttgcttttataaaaaatcattttaagcctttatgctctttaagatcagttttgaaatttcataaacatcatctttgctcatcgccgtaccacttggcaaacaaattcctttttggaaaaataactcactattgccattaagataagccttagttcctttaaatacttcttgagtgtgcatagctttccataatggtcttgtttctatttgttcatttttcaaatcttctatgagttttgaaatttttggatgcaaagtaatatttttttgactgatatttatatctttttgacaagcattaagttcatttttatcaaaatcaatcaaagctgtacttaaccagcgattacttcttgaattttctaattcatctaaaaagctaaaatactctcctaaaaattctttataccactcataaatttctctttttttaagcactctttgttctaaaacctccatttgtgctacaccaatagctcctaaaacattgcttaaacggtaattataaccatagtctaaatgttcataatgcaaacaattttccctagcttgagtgctataaaatcttgctttttcaatcttttctttattttttcctataagcatacctccacctgaagtggtgataattttattgccattataagaataagctccaaattctccaaaagttcctaaggctttattcttataaaaacttcctaaagcttcagcagcatcttcgattaaaacaatttcattttccttgcaaatttcaacaatttcatccattttagccgcattgccataaagatgagttaaaatcaatgcttttggttttttttcacattccttaatagcaagttttaacaaatctacatcgatattataagtttcatcacaatctataaatacaggttttgctttaagataacaaataggcgccactgaagcgataaaagtaaaagaagaagccaaaacaatatcatcttgttttacccctgccacccttaaagctaaatgcaaagctgctgtagctgaatttaaagctaaggcattttcacttttgctataatcttttacactttgctcaaagcgatttacaaattcacccaaaggtgctatataattgcttttgaaaacttcttctatatattttaattcattaccgcccatatgcggaggagaaagaaaaaatctcatgatttatcctttgtataaaacaaaatttttataaattaactctattttacctaaaaaaatttacaaagaatcaaacaaaaatctttttataatcatttcatatttttctttttgcaggcactcccacaaaaacacctttttcattttggcttttaaccaaagttgctccaccacccaaaatactatcatctgctaagcttaaattaggcaaaacacaagaattaatccctaaaaaacaatttttaccgatttttacattacccgcacatttagcccctacgcttacatgagaaaattcccctatcacgcattcatgctcaatcacacttgaagtatttaaaatcacgcctttttctattttggctttagcgttaatcactacatagggcataattaaaatccctgcattttcttccacgcttgcactaggacttataagtgcacttttatgaataagattaactattttaaagccattttctgaaattttttgataaatcttttttcgaatttcattgtttcctatagctataaaaaaatcatatttaggcaaggtgttttcaaatttcattcctttaaaatcatctaaaaaaatacattctttatagcccatatttttagccacatcttcacaaacaagcccatgaccactagcaccataaatataaattttttcagttcttgccattaaatttctctgttgtaacatggccttctttgcttaccccgcttcgttttaaaacctttaaagctgttaaaaacatgatttttaaatcaagcaaaaaagaaatatttttcacataatacacatcaagttcgaattttttctgccaagaaatagcatttctgccatttacctgcgcccatcctgttatacctggacgcaccttatggcgcaatttttgctcttcattataaagggataaatactcaaccaaaagaggtctaggccccacaaaactcatatccccttttaaaacattaaaaagttgcaaaagctcatccaaacttaagcttctaacaatttttccaaaggctttcaaacgcaattcatcgcttaataactcacccttctcatctctttcatcgctcatggttttaaatttataaattttaaaaattttttcatctaacccagggcgattttgagtgaaaatcacacttccttgagtgatttttaaaagtaaagcagtgattaaaatcaccggagaaaaaagtactaaaagcactaaagctaaaataaaatcaaaaattcttttaaaaactttttcatacattcttaattaccctatcataaagttttaaataacgctgtgcgatattattttcatcgtattgtaaagcatcttgggcagcatttttagctaaatttaatcttaatttttcatcttctaataaaagtgaaattttttcgcttaaatccttagcattttttgtttttgcccaaagtccatcataagcattagaaatagcctctacacaaccttcacaatcactcaccactatagccttgccacaagcttttgcctccaaaacacttacaggaaagccttctttatagcttggtaaaacaaaaatatcacaattttgcaaaagctcgactatatcacttctagcacccaaataatgcaccacacccgagtttaaaaactccaaactcgcacaagaaggattttcatctcttccaccaactaaaacaaaatttgctttgtcttttagcatagtagcactttcataaaattcttttacacctttatgccataaagctcttgctatcataagaacaataggttttttatctatatttaaatttctccaaaaaagctcttttttttccgattctatataaataggaaaaaatttttttaaattgatccctacggattttatcacacaaattttattttccttaagtcctaaattccgcataaactcggcattactttcattgacaaaaataaattggtgtgcaaatttaaaacttaatttataaagattattaataacaaaacgtactaaatttgccttaaaaccttgatctatataaaaagatcccaagccttctaccaaagcaaaacgataaggaatttttgcccattttgccgctaaaattccaaaggtattgcttttgtgtgccgcactttgaataagatcaagatttaaattttttaaaaccttagcaagataaaaaaaattctttaaaactacaaaaggatttaaactagctcttgaaaactcataaacaattacttttaaaccaagatctctaagtttttgcgtgtattcatcttgcggcactataacaaaaacttcatcttttctatcttttaatgcttttataataggcattctaaaatgataaatacttgctcctgcatgtgataaaaatcctattctcattttcaacccttaaattttaagtttaaaaaccttagcatctctagaattaatcaccaagtcaaataaattcttatcataatttcctaaaaaaaacatttgcacataagcactattaaacatggttttatccattaaaataaattgtgcgtaaggaatagcactatcctttaaataaaaaatataaaactgagccttatcatcaattggagtgattttgtattcaccttgtttaatagaattaatctctacgatactatttacagaaaccacattatcacctattttaaaacttctaaaatcatcgcttaaaaccactccgttgctaagataaatttctccatttttaacatcaagtggataagctgtgctaaaggtaaaaggtttatccaaaactcctgtatctaaattaataaaagaaaaactagccaccgtagaaaaaatcaaagacattctagcgggcatataaagataaatatcacgagtttttggcgtatcgattttaaaatcaggttttgataatgaagctagaaacaaatccacattgctttgattataatctttcatcatggcttgcaaaatgtctgtttttaaaatatcattttgcggagcataaaagcttttttctgtatattctacactaagtcttgccatattagctgcagcttgttcatctttgcttaaagcaaaagaagggaaaaaattatccttacctaaatgctttccaccatctactaaagttttcacatcgctataataacgcacaggataaccataatcccaccaagttaccacataatcttctctattggctatattttttaattgatttaataatgatgcttcattttgagaaaaaactgttggcgctttatagttgtaaatatggataaatactggagctaaagtcaaaatagttgcaaaaacaatacaaacatttgaagttaattggctatattttttaaccattatagccttaaactcgctcaataaaaaaccaaatcctaaggccattacaggtacagaataaatggtaaatctaagccccccttttaaggctaaaaacccaagcaccaatataggtaaagccataatcatacttttatgttttctcaaaagccatacaaaaccaaacaaagaaaacaaaaaaacaatttcactaccactaattcttcgcataaattcgctaagatctacattttcaacttcttgtatggtttgattgacattaaaatacataaagccctgcgttaaattcgcactttcatcacttctaaaaatataaaatttaagctgataaagtataggatcaaccccaccacttaaaatcaaaaatatcaaagttgcactacctaaaattcctataatcataaaatttaagcgtttttgctctaaggcgaataaagcaaaaagtattactataatggcactttgataaaaccatgctatatttgaaagagtaagagaagacaaaatcacagctatataaaaaatcttttcttttctatgaaaaataagtgtataaattaaaaaaagtccaattaaagctacatttaaagtataacttgaaggataccaccaaagataaattcctataaataacggcaaggcaatcaatgaaaaaaagtctttttttaaaatcattcttaccataaaaaataaaataaacataggcaaaacaattaccagcatatccgtatcataatacccactcatagtgcgattataataactgtttgctatacttgctaaaagagcagctacaaagcccattaaaggacgtttgtattcgttagctagcaaaatagtaggaatcaccaccaaagaagataaaaaagtactcatatataaaatgatactttcaaaagaaaaaggtgtgattttataaagccaataagtaagcgcggataaagaagatccataataactcaaatcattaggctgatgaaaacctgctatcatatctcttgcgccctcagcaaaagcatagccatcatttgaaatgatcattaactgattattgaaaaaatactcattaaactcacttgcccaccaaacccaataaaacctgcaaaatacactaaaaacataagctaatataatcatcgcaaacaaaactaaataagggttttttaaatactcttttttcaacatcttttatcctaataaatatttcaaagcatcgcgtgcaatttttactttatcaaaagctttagccctagttttagccttatttttatacgcttttcttaatttatcgtcttcaagcatagtctttaaaccctgaaacatggagttttcattatctacttctactaaaagtccaaattcatcatcgccaaaaagctctcttgcgccacttttatgatcagtgcaaaccaccgcacaagaacaagctaagctttcaattaaaacatttgaaaagccttcaaatacagaagcaaaagcaaaaaattcgcatttagccatgtatttataaggattattatcaaatcctaaaagcaaaaccttttcttctaaatttaactctttaatcaaagctaaaagctcatctttaagcacaccttcacctaaaatcacaagctttaaatctgttttcaatcttgcataagcacgaattaataaagcatgatttttacctttatcaagcctgcctacacttaaaataaatttatcttttaaagctacatcttcaagagctttttgctctatattttctaaatcgatggcattgtataaaatttcacatttttttggatttatactaaaattttgcactaaatcttctaaatttcccttagaattaggcaagattaaatcagcttttgggtaaagcaaagaaattaaaaatttatttgccaaagaattaaaattatttttcgcatacatcacacttggcgtagtgcattcattgatcacaaggcgagttttgtttccaaacattcttgccattaaggctatataattaggtcgatttaaaaaaacaaattctgtatcaatgcctaaatttctgcaaagttttttatattttaaagccaaaaaaggtagttttaaaaatttcaaaataggattttcactaggttttgaacattctaaaaaatgaatttgacactctggaatttcataagaaattttatcattcattaaaatcaaatgcacttcaaatttcaaacttaaaataggcaataaagtcgccacaactctttcagcaccaccacttcctaaagaataaataaaaatgcctaatttttgcataaagccacccgaatttttgataatttttcaatcatattatttggaattatacttaaaatgagtaatatcaaagcaggagcgttgatttttatactcaggcttttaaacaaacacttataaagagctttataattttttgcaagttttgcataataagctgccattttataataactcgcacaagtttttttataatctttatccttactcattctaagttcattttctaaaattttagcaagctctaaatatcccaaatacaccctatgagcatttttactcgcccctaaagtcacgctatcttgcctaaaaatcctataaatcctaaaagccttatggatataaaaacttttttccttgtataaatttacccaaagcgtggcttcattgccataaaattcttcattaaaacgcttgttttcaagtagagattttttaaaaacagaaaaaaactctccgctaaatttagccattaaaaaatcttttttagaaatttcactatctttttccaagcccttaccgctaaattccttgcttaaatttccttctttttctatcaaacaatttccaaaaacatgagcataaccctcatttgctttttgcatcaaggtacttaaagccccagataaaagctcatcatcatcatctaaaaaagttacaaactcgccacttgcttgatctaagccattgtttttattgccatttgggccttgtttgtaattttgatttaaaaaatacttaatgcgatcatcatctttttgtaaattttgcaccacacttttagtatcatcactagaattatcatcgcttacaatgatttctaaatctttaaaatcttgattttgtatgcttttaatagccttttctaacaaaacttgacgattaaaagttggcactataacagaaagtttaggcatttttaacctcgactataagcttaagccattcttctttgatgttagaaatttcaaagtctttacacctttgtttggcattatttacaagttcttttctaaaattttcatcatttaaaacaagttcaagttttttagcaagtgctatttcatcatcacaacctaccaaaagcccatcatgattatctttgattaaatccttagcaccattataataagaacttgaaattctacaaacctcaaaatacaaactttcaattaaaaccgttggcaaaccctctacaaaagaacaaaggcaaagcacttttgctttttcataaagagccttgacattttcaacgcgtcctaaaaaatcaacttttattcctaaagattttaccttgtattcaagttcttgccttaactctccatctcctgctataacaaatttataattttcttgcaaatttttatccaaatgtgctatagcttttaaaaacattacagggtttttgttgtgatctaaacgccctataaaaagaaccaaattttctttttcaaaactagaatcaaaaggaatttcatcgctaaaatgacaagggtttaataaaagcttaaccctttttacaaatctttcataatacaccttatcactgcttccaagcacacttaaagcatcacaaaaaggatagcttacccttcttaaaaaacgccaagttttaggttttaaatacgcttcattactatgctcgctaatgatgagtggagttttaagtcctatattagctagaatacaagcaatattagttgtatccaaaaaagaaataaaaacatcagccttactttcttttaaagcctttcttaaggcaaaaaatttcttaaaacgacttgcgattttatgataaagcgtgtcaaatctaaattgttctaaacttgtaactttaacttcattttcaagcttataaaaagattctcctgtatgaaatttaataatacttacttcatgctctttgcaaagcgcattagctaaggttactaaaacacgctcagcgcctcctgaatttaaagttgcgataataaagcttattttcatcatttctcctctttaagcttaccgtgttctaaacgataaaccttatcacattgcgttatcgtagaaaggcgatgtgcgataataatcatggttttatctttagaaattttataaatttcatccatgatttttgcttcactttgagtatcaagcgcagaagttgcttcatcaagcactaaaatttcaggctctaaatacaaagcccttgctatagctatgcgttgtttttgtcccccgcttaaattactccccccatcgcctacttttgtctgaactccttgaggtaaattttttataaaatgctctaaatttgcttgtttgataaccttattaagtttttcttcatcaaccgcatctccaaaagtgatatttttagctatgctatcattaaaaagatagatattttgcgggatatagcctattttttggcgataattttttgcattacttgcatttaattcttgcttatcaattaaaatttgcccttcttttggttttaaaagtcctatgataagatctactaaggtactttttccacaaccactctcccctataaaagcgattttttcaccttttttaatgtttaaattaagatttttaaataaatatttttttccctcataaccaaagctaagattgcaaattttaagctcttgattaaaacttaattttccctcgcccaaattttcttcttcttgtcttaaattttgataaataatattcaaagaagaatgataataaagcaaatcatgataacttgtgataatacgatttgcgcttggcattaagcgataaagcgctaaaacaaaaatagaaatcgtggataaaatacctgaaatatcactttcatttttcaaaaccaaaaataccacgataaaaacaagcacacaaaagcctattccttcaagataaattctaggcaccgcagctacgctttcattggtaatatttgctttagaaaaagcttcactttgtgctttaaaaagacttaatactccatcttctttggttttaagcttgataaatttaaaattatttaaatttgtatttaaaatttcgaagaaatttttcatcgcttcttcgcgtcttagtcctgcttttttaatgatagggcttaaaattttcactaaaataaaagcatttaacaccataaaaatacttaaaaataaagtgattttataattaatcaaaagcattaaagcataaagcaaaagcactacaaaaatttcactcatcaaaagtaaaaatgatgaaatcatagtgcttagattataaacttcccctgtaatggactttaaaatttcagattgatttttttgagtaaatttttcataattaatatttaaaaatttagaaaaaaccttataagcgatcgcatgataacgtcctttagaaaatcttgccaaaagatgaaaataatacgcatttaacaaagctctaaatacataaaaaacaataagccccactccaaaataaacaatgatttcaaaaacagggatattaagatattcttttaggctgattaaatatttattacgatcaaaataagaaaaatcactagccaaagtgataaaaggcattaccaaagaaatcgcaaaagtttctataaaagaaacaaatactgaaaaaacaagcaagaaaaataaaaaatttttatcttccttgcttaaaataaaaaaaagtttttt

SEQ ID NO: 42 - DNA, 2133 bp, Campylobacter sputorum
atgagtaattttaattttgccaaatttctgaacaagctgcctagactaagcaaacataccatcctgatgatcgtgctggcggtgtgctttggcatcttttgtcgcttttattgggttgtgtgggcgagtgcgtatccacattttatttggaatgatgaactgatgatctctacaaatgatggctatgcgtttgcggaaggtacacgcgatatgattgccggctttcatcagccgaatgatctgtcatattatggtcgttcactgtccactttaagcatgtggctgtatagcatcctgccgttttcattagaaaccatcttactgtatatgtcaacgtttctgagtccactgctggcagttccgttaatcttaatcggtaaagaactgaatgcgtctaaagcaggctttattgcagccctgctggcagttgtggccaatagctattataatcgcaccatgtcaggctattatgatacggatatgctgaatatcaccttaccgatgatggtgttttggagcatcacccgcctggttcagcgcaaagaacgggttaatctcatctttattccagtgtttatggccatctatggttggtggtatccatcttcatattcactgctgctggccatgatcggcatgtttgtgctgtataccatcgtgtttgaacgctatgaaaaactgaattatgaagcaatggtgtttatgattctggcaatcactagctttccgattcagatcaagtttatcatcgtgatcattctgtatgcgttaatctatttttatcagcgctttttcgataaaaaagttatctttgccttaatcattgcaagtagcatttgctttatttggttaggcggcttaaatccaatcctgtttcctatcaaattttatatctttcgcgacatagcggattcaggcgatacggtgtttaaattcttcaatgtggttcagaccattcgcgaaagtagcgccatcgattttaatacagttgcgacccgcatctcaggtcatctgattgtgtttctggtgagcatcgtgggctatatcctgtttatcaaaaacaacaagattttactgctgaccttaccgatcctgtttctgggtctgatgtcgtttaaaagcggcctgcgctttacaatctatagcgttcctgtaatggcgttaggctttggctattttgtgatgtattgctttacgaaaatcgacatcaaagatcgctttctgggctatgcctttctgtttgtggtgacctttagtgccctgtatccgtcactgaaacatatctatgattacaaggtgtttccagtgtttacacatagcgaagtggaaagcctggatgatctgaaaaatattgccaaacgcgaagattatgtgctgtcttggtgggattatggctatccgattcgctattatagcgatgttaaaacactgatcgatggcggtaaacatctaggttcagataattttgccgtgagctttgcactgggcagcgatcagaatagtagtgcaaatatggcccgcttagaagtggaatatacggaacgcaattatgaagaaaaatttggtctgaatctgaaacagatcatgaaagattataatgcaaccaatgtgaatgagtttctgctgtctctgaaagatgccaacctggccctgcctaaacagacacgcgatatatattattatctgccggatcgcatgatctatatctatcctacagtgttagcctttagtcgcctggatctgacgacgggccaggaatttgcagaaccgtttttcatcgtgagcgaacgctttagtgcaaccaatgataatcagatcatgttaaacaacaatgtgattctttcatcagatggaacaaaactgtcaatcaatggcaatagctattcagttaatacttatgtagaaaccagctacgatcagaacgaaaaactgaatgttaattattttaatatcgatccgaatagcaatttttatgtgatctttatgaaagattatctgcgcatcttagttctggataaaaccctgtatgatagcgcgtatatccagctgtttgtgctggaaaattatgataaaaatctgtttgaaccagtcatcctgaatggtagtacgaaaatctataagctgaaaaaataa

SEQ ID NO: 43 - protein, 710 aa, Campylobacter sputorum
MSNFNFAKFLNKLPRLSKHTILMIVLAVCFGIFCRFYWVVWASAYPHFIWNDELMISTNDGYAFAEGTRDMIAGFHQPNDLSYYGRSLSTLSMWLYSILPFSLETILLYMSTFLSPLLAVPLILIGKELNASKAGFIAALLAVVANSYYNRTMSGYYDTDMLNITLPMMVFWSITRLVQRKERVNLIFIPVFMAIYGWWYPSSYSLLLAMIGMFVLYTIVFERYEKLNYEAMVFMILAITSFPIQIKFIIVIILYALIYFYQRFFDKKVIFALIIASSICFIWLGGLNPILFPIKFYIFRDIADSGDTVFKFFNVVQTIRESSAIDFNTVATRISGHLIVFLVSIVGYILFIKNNKILLLTLPILFLGLMSFKSGLRFTIYSVPVMALGFGYFVMYCFTKIDIKDRFLGYAFLFVVTFSALYPSLKHIYDYKVFPVFTHSEVESLDDLKNIAKREDYVLSWWDYGYPIRYYSDVKTLIDGGKHLGSDNFAVSFALGSDQNSSANMARLEVEYTERNYEEKFGLNLKQIMKDYNATNVNEFLLSLKDANLALPKQTRDIYYYLPDRMIYIYPTVLAFSRLDLTTGQEFAEPFFIVSERFSATNDNQIMLNNNVILSSDGTKLSINGNSYSVNTYVETSYDQNEKLNVNYFNIDPNSNFYVIFMKDYLRILVLDKTLYDSAYIQLFVLENYDKNLFEPVILNGSTKIYKLKK

SEQ ID NO: 44 - DNA, 2142 bp, Campylobacter jejuni
atgttgaaaaaagagtatttaaaaaacccttatttagttttgtttgcgatgattatattagcttatgtttttagtgtattttgcaggttttattgggtttggtgggcaagtgagtttaatgagtattttttcaataatcagttaatgatcatttcaaatgatggctatgcttttgctgagggcgcaagagatatgatagcaggttttcatcagcctaatgatttgagttattatggacgttctttatccgcgcttacttattggctttataaaatcacacctttttcttttgaaagtatcattttatatatgagtacttttttatcttctttggtggtgattcctactattttgctagctaacgaatacaaacgtcctttaatgggctttgtagctgctcttttagcaagtatagcaaacagttattataatcgcactatgagtgggtattatgatacggatatgctggtaattgttttgcctatgtttattttattttttatggtaagaatgattttaaaaaaagactttttttcattgattgccttgccgttatttataggaatttatctttggtggtatccttcaagttatactttaaatgtagctttaattggactttttttaatttatacacttatttttcatagaaaagaaaagattttttatatagctgtgattttgtcttctcttactctttcaaatatagcatggttttatcaaagtgccattatagtaatactttttgctttattcgccttagagcaaaaacgcttaaattttatgattataggaattttaggtagtgcaactttgatatttttgattttaagtggtggggttgatcctatactttatccgcttaaattttatatttttagaagtgatgaaagtgcgaatttaacgcagggctttatgtattttaatgtcgttcaaaccatacaagaagttgaaaatgtagatcttagcgaatttatgcgaagaattagtggtagtgaaattgtttttttgttttctttgtttggttttgtatggcttttgagaaaacataaaagtatgattatggctttacctatattggtgcttgggtttttagccttaaaaggggggcttagatttaccatttattctgtacctgtaatggccttaggatttggttttttattgagcgagtttaaggctataatggttaaaaaatatagccaattaacttcaaatgtttgtattgtttttgcaactattttgactttagctccagtatttatccatatttacaactataaagcgccaacagttttttctcaaaatgaagcatcattattaaatcaattaaaaaatatagccaatagagaagattatgtggtaacttggtgggattatggttatcctgtgcgttattatagcgatgtgaaaactttagtagatggtggaaagcatttaggtaaggataattttttcccttcttttgctttaagcaaagatgaacaagctgcagctaatatggcaagacttagtgtagaatatacagaaaaaagcttttatgctccgcaaaatgatattttaaaaacagacattttgcaagccatgatgaaagattataatcaaagcaatgtggatttgtttctagcttcattatcaaaacctgattttaaaatcgatacgccaaaaactcgtgatatttatctttatatgcccgctagaatgtctttgattttttctacggtggctagtttttcttttattaatttagatacaggagttttggataaaccttttacctttagcacagcttatccacttgatgttaaaaatggagaaatttatcttagcaacggagtggttttaagcgatgattttagaagttttaaaataggtgataatgtggtttctgtaaatagtatcgtagagattaattctattaaacaaggtgaatacaaaatcactccaattgatgataaggctcagttttatattttttatttaaaggatagtgctattccttacgcacaatttattttaatggataaaaccatgtttaatagtgcttatgtgcaaatgttttttttaggaaattatgataagaatttatttgacttggtgattaattctagagatgctaaggtttttaaacttaaaatttaa

SEQ ID NO: 45 - protein, 713 aa, Campylobacter jejuni
MLKKEYLKNPYLVLFAMIILAYVFSVFCRFYWVWWASEFNEYFFNNQLMIISNDGYAFAEGARDMIAGFHQPNDLSYYGRSLSALTYWLYKITPFSFESIILYMSTFLSSLVVIPTILLANEYKRPLMGFVAALLASIANSYYNRTMSGYYDTDMLVIVLPMFILFFMVRMILKKDFFSLIALPLFIGIYLWWYPSSYTLNVALIGLFLIYTLIFHRKEKIFYIAVILSSLTLSNIAWFYQSAIIVILFALFALEQKRLNFMIIGILGSATLIFLILSGGVDPILYPLKFYIFRSDESANLTQGFMYFNVVQTIQEVENVDLSEFMRRISGSEIVFLFSLFGFVWLLRKHKSMIMALPILVLGFLALKGGLRFTIYSVPVMALGFGFLLSEFKAIMVKKYSQLTSNVCIVFATILTLAPVFIHIYNYKAPTVFSQNEASLLNQLKNIANREDYVVTWWDYGYPVRYYSDVKTLVDGGKHLGKDNFFPSFALSKDEQAAANMARLSVEYTEKSFYAPQNDILKTDILQAMMKDYNQSNVDLFLASLSKPDFKIDTPKTRDIYLYMPARMSLIFSTVASFSFINLDTGVLDKPFTFSTAYPLDVKNGEIYLSNGVVLSDDFRSFKIGDNVVSVNSIVEINSIKQGEYKITPIDDKAQFYIFYLKDSAIPYAQFILMDKTMFNSAYVQMFFLGNYDKNLFDLVINSRDAKVFKLKI